European Patent Application EP 4 806 911 A1, published September 16, 2026. Title: TRIPLE AGONIST COMPOUND. Applicant: Chengdu Aoda Biotechnology CO.,Ltd. The sequence listing filed with the application follows.

SEQUENCE LISTING (13 sequences)

SEQ ID NO: 1 - protein, 39 aa, synthetic construct
  MOD_RES 2: note = X is Aib
  MOD_RES 13: note = X is alpha MeLeu
  MOD_RES 17: note = X is Lys(2-(2-aminoethoxy) ethoxyacetic acid-gamma Glu-eicosanedioic acid)
  MOD_RES 20: note = X is Aib
YXQGTFTSDYSIXLDKXAQXAFIEYLLEGGPSSGAPPPS

SEQ ID NO: 2 - protein, 39 aa, synthetic construct
  MOD_RES 2: note = X is Aib
  MOD_RES 6: note = X is alpha-MePhe
  MOD_RES 13: note = X is alpha-MeLeu
  MOD_RES 17: note = X is Lys(2-(2-aminoethoxy) ethoxyacetic acid-Gamma Glu-eicosanedioic acid)
  MOD_RES 20: note = X is Aib
YXQGTXTSDYSIXLDKXAQXAFIEYLLEGGPSSGAPPPS

SEQ ID NO: 3 - protein, 39 aa, synthetic construct; identical to SEQ ID NO: 2
  MOD_RES 2: note = X is Aib
  MOD_RES 6: note = X is alpha-MePhe
  MOD_RES 13: note = X is alpha-MeLeu
  MOD_RES 17: note = X is Lys(2-(2-aminoethoxy) ethoxyacetic acid-Delta Aad-eicosanedioic acid)
  MOD_RES 20: note = X is Aib

SEQ ID NO: 4 - protein, 39 aa, synthetic construct; identical to SEQ ID NO: 2
  MOD_RES 2: note = X is Aib
  MOD_RES 6: note = X is alpha-MePhe
  MOD_RES 13: note = X is alpha-MeLeu
  MOD_RES 17: note = X is Lys(2-(2-aminoethoxy) ethoxyacetic acid-Epsilon Apm-eicosanedioic acid)
  MOD_RES 20: note = X is Aib

SEQ ID NO: 5 - protein, 39 aa, synthetic construct; identical to SEQ ID NO: 2
  MOD_RES 2: note = X is Aib
  MOD_RES 6: note = X is alpha-MePhe
  MOD_RES 13: note = X is alpha-MeLeu
  MOD_RES 17: note = X is Lys(2-(2-aminoethoxy) ethoxyacetic acid-Zeta Asu-eicosanedioic acid)
  MOD_RES 20: note = X is Aib

SEQ ID NO: 6 - protein, 39 aa, synthetic construct; identical to SEQ ID NO: 2
  MOD_RES 2: note = X is Aib
  MOD_RES 6: note = X is alpha-MePhe(2F)
  MOD_RES 13: note = X is alpha-MeLeu
  MOD_RES 17: note = X is Lys(2-(2-aminoethoxy) ethoxyacetic acid-Gamma Glu-eicosanedioic acid)
  MOD_RES 20: note = X is Aib

SEQ ID NO: 7 - protein, 39 aa, synthetic construct; identical to SEQ ID NO: 2
  MOD_RES 2: note = X is Aib
  MOD_RES 6: note = X is alpha-MePhe(2F)
  MOD_RES 13: note = X is alpha-MeLeu
  MOD_RES 17: note = X is Lys(2-(2-aminoethoxy) ethoxyacetic acid-Delta Aad-eicosanedioic acid)
  MOD_RES 20: note = X is Aib

SEQ ID NO: 8 - protein, 39 aa, synthetic construct; identical to SEQ ID NO: 2
  MOD_RES 2: note = X is Aib
  MOD_RES 6: note = X is alpha-MePhe(2F)
  MOD_RES 13: note = X is alpha-MeLeu
  MOD_RES 17: note = X is Lys(2-(2-aminoethoxy) ethoxyacetic acid-Epsilon Apm-eicosanedioic acid)
  MOD_RES 20: note = X is Aib

SEQ ID NO: 9 - protein, 39 aa, synthetic construct; identical to SEQ ID NO: 2
  MOD_RES 2: note = X is Aib
  MOD_RES 6: note = X is alpha-MePhe(2F)
  MOD_RES 13: note = X is alpha-MeLeu
  MOD_RES 17: note = X is Lys(2-(2-aminoethoxy) ethoxyacetic acid-Zeta Asu-eicosanedioic acid)
  MOD_RES 20: note = X is Aib

SEQ ID NO: 10 - protein, 39 aa, synthetic construct; identical to SEQ ID NO: 2
  MOD_RES 2: note = X is Aib
  MOD_RES 6: note = X is alpha-MePhe
  MOD_RES 13: note = X is alpha-MeLeu
  MOD_RES 17: note = X is Lys(2-(2-aminoethoxy) ethoxyacetic acid-2-(2-aminoethoxy) ethoxyacetic acid-Gamma Glu-eicosanedioic acid)
  MOD_RES 20: note = X is Aib

SEQ ID NO: 11 - protein, 39 aa, synthetic construct; identical to SEQ ID NO: 2
  MOD_RES 2: note = X is Aib
  MOD_RES 6: note = X is alpha-MePhe
  MOD_RES 13: note = X is alpha-MeLeu
  MOD_RES 17: note = X is Lys(COCH2PEG5-Gamma Glu-eicosanedioic acid)
  MOD_RES 20: note = X is Aib

SEQ ID NO: 12 - protein, 39 aa, synthetic construct; identical to SEQ ID NO: 2
  MOD_RES 2: note = X is Aib
  MOD_RES 6: note = X is alpha-MePhe(2F)
  MOD_RES 13: note = X is alpha-MeLeu
  MOD_RES 17: note = X is Lys(2-(2-aminoethoxy) ethoxyacetic acid-2-(2-aminoethoxy) ethoxyacetic acid-Gamma Glu-eicosanedioic acid)
  MOD_RES 20: note = X is Aib

SEQ ID NO: 13 - protein, 39 aa, synthetic construct; identical to SEQ ID NO: 2
  MOD_RES 2: note = X is Aib
  MOD_RES 6: note = X is alpha-MePhe(2F)
  MOD_RES 13: note = X is alpha-MeLeu
  MOD_RES 17: note = X is Lys(COCH2PEG5-Gamma Glu-eicosanedioic acid)
  MOD_RES 20: note = X is Aib